European Patent Application EP 4 385 518 A1, published June 19, 2024. Title: Kit for combination therapy of tumor diseases and/or infections. Applicant: Julius-Maximilians-Universität Würzburg. The sequence listing filed with the application follows.

SEQUENCE LISTING (5 sequences)

SEQ ID NO: 1 - protein, 518 aa, Aplysia punctata
MDGVSRNRRQCNREVCGSTYDVAVVGAGPGGANSAYMLRDSGLDIAVFEYSDRVGGRLFTYQLPNTPDVNLEIGGMRFIEGAMHRLWRVISELGLTPKVFKEGFGKEGRQRFYLRGQSLTKKQVKSGDVPYDLSPEEKENQGNLVEYYLEKLTGLQLNGEPLKREVALKLTVPDGRFLYDLSFDEAMDLVASPEGKEFTRDTHVFTGEVTLDASAVSLFDDHLGEDYYGSEIYTLKEGLSSVPQGLLQAFLDAADSNEFYPNSHLKALRRKTNGQYVLYFEPTTSKDGQTTINYLEPLQVVCAQRVILAMPVYALNQLDWNQLRNDRATQAYAAVRPIPASKVFMTFDQPWWLENERKSWVTKSDALFSQMYDWQKSEASGDYILIASYADGLKAQYLRELKNQGEDIPGSDPGYNQVTEPLKDTILDHLTEAYGVERDSIPEPVTAASQFWTDYPFGCGWITWRAGFHFDDVISTMRRPSLKDEVYVVGADYSWGLISSWIEGALETSENVINDYFL

SEQ ID NO: 2 - protein, 64 aa, synthetic construct
VDNKFNKEMRNAYWEIALLPNLNNQQKRAFIRSLYDDPSQSANLLAEAKKLNDAQAPKGGSGGS

SEQ ID NO: 3 - protein, 64 aa, synthetic construct
VDNRFNAEMRNAYWEIALLPNLNNQQRRAFIRSLYDDPSQSANLLAEARALNDAQAPAGGSGGS

SEQ ID NO: 4 - protein, 589 aa, synthetic construct
MVDNRFNAEMRNAYWEIALLPNLNNQQRRAFIRSLYDDPSQSANLLAEARALNDAQAPAGGGSGGGDGGGSMDGVSRNRRQCNREVCGSTYDVAVVGAGPGGANSAYMLRDSGLDIAVFEYSDRVGGRLFTYQLPNTPDVNLEIGGMRFIEGAMHRLWRVISELGLTPKVFKEGFGKEGRQRFYLRGQSLTKKQVKSGDVPYDLSPEEKENQGNLVEYYLEKLTGLQLNGEPLKREVALKLTVPDGRFLYDLSFDEAMDLVASPEGKEFTRDTHVFTGEVTLDASAVSLFDDHLGEDYYGSEIYTLKEGLSSVPQGLLQAFLDAADSNEFYPNSHLKALRRKTNGQYVLYFEPTTSKDGQTTINYLEPLQVVCAQRVILAMPVYALNQLDWNQLRNDRATQAYAAVRPIPASKVFMTFDQPWWLENERKSWVTKSDALFSQMYDWQKSEASGDYILIASYADGLKAQYLRELKNQGEDIPGSDPGYNQVTEPLKDTILDHLTEAYGVERDSIPEPVTAASQFWTDYPFGCGWITWRAGFHFDDVISTMRRPSLKDEVYVVGADYSWGLISSWIEGALETSENVINDYFL

SEQ ID NO: 5 - protein, 589 aa, synthetic construct; identical to SEQ ID NO: 4